European Patent Specification EP 3 404 088 B1, published March 5, 2025. Title: DETERGENT COMPOSITION COMPRISING A VARIANT OF A FAMILY 44 XYLOGLUCANASE VARIANTs. Applicant: THE PROCTER AND GAMBLE COMPANY. The sequence listing filed with the application follows.

SEQUENCE LISTING (7 sequences)

SEQ ID NO: 1 - DNA, 1695 bp, Paenibacillus polymyxa
atgaagaaaccgttggggaaaattgtcgcaagcaccgcactactcatttctgttgcttttagttcatcgatcgcatcggctgtagttcacggtcaaacggcaaagactattactattaaagtagatacattcaaggatcgtaagcctattagcccttatatatacggtacaaatcaggatttggcaggcgatgaaaatatggctgccagacgacttggtggcaaccgaatgaccggatacaactgggaaaacaatatgtccaatgcaggaagtgactggcagcaatctagcgataactatttatgcagtaatggtggcctgacacaagccgaatgtgaaaagccaggagcggtgacgacttcgtttcatgaccaatcgctgaagcttggcacttattctttagttacgttgccgatggccggttatgtggctaaggatggaaacggaagtgtgcaggaaagcgaaaaggccccttccgctcgttggaatcaggtcgtaaacgccaaaaatgcaccgttccaactacagcctgatctgaatgacaatcgggtctatgtggatgagttcgtccattttttagtgaacaagtacggcactgcttcaacaaaggcgggggtgaaaggatatgccctcgacaatgaacccgctctctggtcgcatacgcacccacgcattcatggtgaaaaagtcggagcgaaagagttggtagaccggtcagtcagtttatccaaagctgtgaaagcgattgacgcgggggcagaggtttttggcccggttctttacggatttggcgcctataaagatcttcaaactgcacctgattgggactctgtaaaaggcaattatagctggttcgtagactattacctggatcaaatgcgccttagctcgcaagtcgaaggcaagagattgctggatgtattcgacgtacactggtatcccgaagcgatgggcggaggcatacgaattacgaatgaggtaggcaatgacgaaacgaagaaagccagaatgcaggcacctcgcaccttgtgggacccgacctataaggaagatagttggatcgctcaatggaacagcgagtttttgcccatactacctcgattgaagcagtcggtggataaatattatccgggaaccaagctggcaatgaccgagtatagctatggcggcgaaaatgatatttccggcgggattgcgatgaccgatgtgctgggtatcttgggcaaaaatgatgtttatatggcaaactactggaagctaaaggatggtgtcaacaactacgttagtgccgcttacaagctttatcgcaattatgacggaaaaaactctactttcggtgataccagtgttagtgcgcaaacatcggatattgtcaatagctcggtccatgcttctgtaacgaatgcatccgacaaagaactgcatctcgttgtcatgaataaaagcatggacagcgcattcgacgcccaatttgatctttccggcgcgaagacttacatttccggtaaagtatgggggttcgataaaaacagctcgcaaattaaagaagcagcgccaatcacgcaaatttcaggcaaccgttttacttataccgtaccgcctttgacggcatatcacattgtgctgactactggcaatgacacgtctccagtgtaaggcgtacttgtttggggaaccgagccgacagctaattaa

SEQ ID NO: 2 - protein, 551 aa, Paenibacillus polymyxa
MKKPLGKIVASTALLISVAFSSSIASAVVHGQTAKTITIKVDTFKDRKPISPYIYGTNQDLAGDENMAARRLGGNRMTGYNWENNMSNAGSDWQQSSDNYLCSNGGLTQAECEKPGAVTTSFHDQSLKLGTYSLVTLPMAGYVAKDGNGSVQESEKAPSARWNQVVNAKNAPFQLQPDLNDNRVYVDEFVHFLVNKYGTASTKAGVKGYALDNEPALWSHTHPRIHGEKVGAKELVDRSVSLSKAVKAIDAGAEVFGPVLYGFGAYKDLQTAPDWDSVKGNYSWFVDYYLDQMRLSSQVEGKRLLDVFDVHWYPEAMGGGIRITNEVGNDETKKARMQAPRTLWDPTYKEDSWIAQWNSEFLPILPRLKQSVDKYYPGTKLAMTEYSYGGENDISGGIAMTDVLGILGKNDVYMANYWKLKDGVNNYVSAAYKLYRNYDGKNSTFGDTSVSAQTSDIVNSSVHASVTNASDKELHLVVMNKSMDSAFDAQFDLSGAKTYISGKVWGFDKNSSQIKEAAPITQISGNRFTYTVPPLTAYHIVLTTGNDTSPV

SEQ ID NO: 3 - protein, 524 aa, Paenibacillus polymyxa
VVHGQTAKTITIKVDTFKDRKPISPYIYGTNQDLAGDENMAARRLGGNRMTGYNWENNMSNAGSDWQQSSDNYLCSNGGLTQAECEKPGAVTTSFHDQSLKLGTYSLVTLPMAGYVAKDGNGSVQESEKAPSARWNQVVNAKNAPFQLQPDLNDNRVYVDEFVHFLVNKYGTASTKAGVKGYALDNEPALWSHTHPRIHGEKVGAKELVDRSVSLSKAVKAIDAGAEVFGPVLYGFGAYKDLQTAPDWDSVKGNYSWFVDYYLDQMRLSSQVEGKRLLDVFDVHWYPEAMGGGIRITNEVGNDETKKARMQAPRTLWDPTYKEDSWIAQWNSEFLPILPRLKQSVDKYYPGTKLAMTEYSYGGENDISGGIAMTDVLGILGKNDVYMANYWKLKDGVNNYVSAAYKLYRNYDGKNSTFGDTSVSAQTSDIVNSSVHASVTNASDKELHLVVMNKSMDSAFDAQFDLSGAKTYISGKVWGFDKNSSQIKEAAPITQISGNRFTYTVPPLTAYHIVLTTGNDTSPV

SEQ ID NO: 4 - DNA, 1590 bp, Paenibacillus polymyxa
gtagttcacggtcaaacggcaaagactgttaccattaaagtcgatacatccaaggatcgtaagcctattagcccttatatttacggtacgaatcaggagttggcaggcgatgagaatctgactgccagacgacttggtggcaatcgaatgaccggatataactgggaaaacaatatgtccaatgcaggaagcgactggatgcagtccagcgatagctatttatgcgacaacgccggattgacaaaagccgaatgtgaaaagccaggtgcggtggcaacctcgtttcacgatcaatcgctgaagcagggcacatattctttagtcacactgccgatggccggttatgtggccaaggatggaaacggaagtgtgcaggaaagcgaaaaggctccttccgctcggtggaatgaggtcgtaaacgctaaaaatgcgccgtttcaattgcagcctgatctgaaagacaatcaggtttatgcggatgaattcgtcaactttttagtgaaaaagtacggcgttgcttcaacaaaaacgggcgtgaaaggatactcgctcgacaatgaacccgctctctggtcgcatacgcatccgcgcattcatggtgaaaaggtcggagcgaaagagttggtagaccggtcggtaagtttatccaaagccgctaaggcggttgacgcgggtgcggaaatttttgggcccgttctttacggttttggcgcctataaagatcttcaaactgcacctgattggaactctgtaaaaggcaactacagctggttcgtggactattacctcgatcaaatgcgcctcagctcgcaagccgaaggcaagagattgctggatgtcttcgatgtacactggtatcctgaagcgatgggcggaggcatacgaattacaaatgaggtaggcaacgacgaaacgaagaaagccagaatgcaagcgcctcgtactttgtgggatccgacctacaaggaagatagctggatcgctcaatggaacagtgaattcttgcctttactgcctcgattaaagcagtcggtggataagtattacccgggaaccaagctggctttgactgagtatagctatggtggcgaaaatgatatttccggcggtatcgctatggccgatgtgctgggcatcttgggcaaaaacgacgtttatatggcaaactactggaagttaaaggatggtgccaacaactacgttagtgccgcttacaagctttaccgcaattatgacggaaaaagctctactttcggtgatatcagcgttcatgcgcaaacgtcggatattgttaatagctcggtgcatgcttccgtaacggatgcatcctacaaagaactgcacctcgttgtcatgaataaaagcatggacagtgcattcgacgcccaatttgatctttccggcgagacgacttacggttccggtaaagtatggggtttcgacaaaaatagctcgcaaattaaggaagcagcgccaatcacscaaatttcaggcaaccgytttacctatacagtaccgcctttgacggcttatcacatcgtgttgactgccggcaatgatacacctgtagaaaatcctgaaagctttgcg

SEQ ID NO: 5 - protein, 530 aa, Paenibacillus polymyxa
VVHGQTAKTVTIKVDTSKDRKPISPYIYGTNQELAGDENLTARRLGGNRMTGYNWENNMSNAGSDWMQSSDSYLCDNAGLTKAECEKPGAVATSFHDQSLKQGTYSLVTLPMAGYVAKDGNGSVQESEKAPSARWNEVVNAKNAPFQLQPDLKDNQVYADEFVNFLVKKYGVASTKTGVKGYSLDNEPALWSHTHPRIHGEKVGAKELVDRSVSLSKAAKAVDAGAEIFGPVLYGFGAYKDLQTAPDWNSVKGNYSWFVDYYLDQMRLSSQAEGKRLLDVFDVHWYPEAMGGGIRITNEVGNDETKKARMQAPRTLWDPTYKEDSWIAQWNSEFLPLLPRLKQSVDKYYPGTKLALTEYSYGGENDISGGIAMADVLGILGKNDVYMANYWKLKDGANNYVSAAYKLYRNYDGKSSTFGDISVHAQTSDIVNSSVHASVTDASYKELHLVVMNKSMDSAFDAQFDLSGETTYGSGKVWGFDKNSSQIKEAAPITQISGNRFTYTVPPLTAYHIVLTAGNDTPVENPESFA

SEQ ID NO: 6 - DNA, 1575 bp, Paenibacillus polymyxa
gtggttcacggtcaaacggcaaagaccgttaccattaaagtcgatacatccaaggatcgtaagcctattagtccttatatatacggtacgaatcaggatttggcaggcgatgaaaatctggctgccagacgacttggtggcaatcgaatgaccggatacaactgggaaaataatatgtccaatgcgggaagcgattggcagcaatccagcgataactttttatgcaacaatggtggcctgacaaaagccgaatgtgaaaagccgggagcagtgacgacttcgtttcatgatcaatcgctgaagctgggcgcttattctttagtcacgctgccgatggccggttatgtggccaaggatggaaacggaagtgtgcaggaaagcgaacaggctccttccgctcgttggaatcaggtcgtaaatgccaaaaatgcgccgttccaactacagcctgatctgaatgacaatcaggtatatgcggatgaattcgtcaattttttagtgaaaaagtacggcgctgcttcaacaaaggcgggtgtgaaaggatatgcgctcgacaatgaacccgctctctggtcgcatacgcatccgcgcattcatggtgaaaaggtcggagcgaaagagttggtagaccggtcggtaagtttatccaaagctgttaaagcggttgacgcgggtgcagaaatttttgggccggttctttacggttttggcgcctatacagatcttcaaactgcacctgattggaactctgtaaaaggcaactatagctggttcgtggactattacctggatcaaatgcgcctcaactcgcaagccgarggcaagagattgctggaygtattcgatgtgcactggtatcccgaagcgatgggcggaggcatacgaattacaaatgaggtaggcaatgacgaaacgaagaaagccagaatgcaggcgcctcgtactttgtgggacccgacctacaaggaagatagctggatcgctcaatggaacagcgcattcttgcctttactgcctcgattgaagcagtcggtggacaagtattacccgggaaccaagctggctttgaccgagtatagctacggcggcgaaaatgatatttccggcggtattgctatgaccgatgtgctgggcatcttgggcaaaaacgacgtttatatggcgaactattggaagttaaaggatggtgccaacaactacgttagcgccgcttacaagctttaccgcaattatgacggaaaaaacgctactttcggcgatatcagcgttaatgcgcaaacgtcggatattgttaatagctcggtgcatgcttccgtaacggatgcatcctacaaagaactgcacctcattgtcatgaataaaagcatggacagcgcattcgacgcccaattcgatctttccggcgagacgacttacagttccggtaaaatatggggcttcgataaaaatagctcgcaaattaaggcagtagcgccaatcacgcaaatttcaggcaaccgctttacctatacagtaccacctttgacggcttatcacatcgtgttgactgccgacaatgatacacctgtgccataa

SEQ ID NO: 7 - protein, 524 aa, Paenibacillus polymyxa
VVHGQTAKTVTIKVDTSKDRKPISPYIYGTNQDLAGDENLAARRLGGNRMTGYNWENNMSNAGSDWQQSSDNFLCNNGGLTKAECEKPGAVTTSFHDQSLKLGAYSLVTLPMAGYVAKDGNGSVQESEQAPSARWNQVVNAKNAPFQLQPDLNDNQVYADEFVNFLVKKYGAASTKAGVKGYALDNEPALWSHTHPRIHGEKVGAKELVDRSVSLSKAVKAVDAGAEIFGPVLYGFGAYTDLQTAPDWNSVKGNYSWFVDYYLDQMRLNSQAEGKRLLDVFDVHWYPEAMGGGIRITNEVGNDETKKARMQAPRTLWDPTYKEDSWIAQWNSAFLPLLPRLKQSVDKYYPGTKLALTEYSYGGENDISGGIAMTDVLGILGKNDVYMANYWKLKDGANNYVSAAYKLYRNYDGKNATFGDISVNAQTSDIVNSSVHASVTDASYKELHLIVMNKSMDSAFDAQFDLSGETTYSSGKIWGFDKNSSQIKAVAPITQISGNRFTYTVPPLTAYHIVLTADNDTPVP